European Patent Application EP 4 745 249 A1, published May 20, 2026. Title: １種以上のＨＬＡ－ＤＰ遺伝子用プライマー. Applicant: National Center for Global Health and Medicine. Application JP. The sequence listing filed with the application follows.

SEQUENCE LISTING (22 sequences)

SEQ ID NO: 1 - DNA, 17 bp, synthetic construct
  misc_feature 1..17: note = Forward primer for HLA-DPA1 gene
  source 1..17: mol_type = other DNA
aacctatccccctccct

SEQ ID NO: 2 - DNA, 20 bp, synthetic construct
  misc_feature 1..20: note = Forward primer for HLA-DPA1 gene
  source 1..20: mol_type = other DNA
aaacctatccccctccctcc

SEQ ID NO: 3 - DNA, 14 bp, synthetic construct
  misc_feature 1..14: note = Reverse primer for HLA-DPA1 gene
  source 1..14: mol_type = other DNA
atctgacctggaaa

SEQ ID NO: 4 - DNA, 20 bp, synthetic construct
  misc_feature 1..20: note = Reverse primer for HLA-DPA1 gene
  source 1..20: mol_type = other DNA
gccatctgacctggaaacca

SEQ ID NO: 5 - DNA, 14 bp, synthetic construct
  misc_feature 1..14: note = Forward primer for HLA-DPA1 gene
  source 1..14: mol_type = other DNA
actgtacccatgtc

SEQ ID NO: 6 - DNA, 24 bp, synthetic construct
  misc_feature 1..24: note = Forward primer for HLA-DPA1 gene
  source 1..24: mol_type = other DNA
tttactgtacccatgtccttggag

SEQ ID NO: 7 - DNA, 17 bp, synthetic construct
  misc_feature 1..17: note = Reverse primer for HLA-DPA1 gene
  source 1..17: mol_type = other DNA
cagaacccagaaagatt

SEQ ID NO: 8 - DNA, 24 bp, synthetic construct
  misc_feature 1..24: note = Reverse primer for HLA-DPA1 gene
  source 1..24: mol_type = other DNA
cctcagaacccagaaagattcaga

SEQ ID NO: 9 - DNA, 16 bp, synthetic construct
  source 1..16: mol_type = other DNA
tcagatgctttgaagg

SEQ ID NO: 10 - DNA, 24 bp, synthetic construct
  source 1..24: mol_type = other DNA
agaatcagatgctttgaaggaggt

SEQ ID NO: 11 - DNA, 16 bp, synthetic construct
  source 1..16: mol_type = other DNA
gccagaggtctcatta

SEQ ID NO: 12 - DNA, 24 bp, synthetic construct
  source 1..24: mol_type = other DNA
gagtcttgccagaggtctcattaa

SEQ ID NO: 13 - DNA, 15 bp, synthetic construct
  source 1..15: mol_type = other DNA
cgcccatattttgat

SEQ ID NO: 14 - DNA, 24 bp, synthetic construct
  source 1..24: mol_type = other DNA
tgcgcccatattttgatcttgttt

SEQ ID NO: 15 - DNA, 13 bp, synthetic construct
  source 1..13: mol_type = other DNA
gaactaggggaca

SEQ ID NO: 16 - DNA, 24 bp, synthetic construct
  source 1..24: mol_type = other DNA
attgtgaactaggggacatttgga

SEQ ID NO: 17 - DNA, 15 bp, synthetic construct
  source 1..15: mol_type = other DNA
agagaggcagtgtcg

SEQ ID NO: 18 - DNA, 20 bp, synthetic construct
  source 1..20: mol_type = other DNA
ccaagagaggcagtgtcgtt

SEQ ID NO: 19 - DNA, 60 bp, Homo sapiens
  source 1..60: mol_type = genomic DNA
ggagcagccgggttggcctaagggaccttagtgccgggcggaaaggggactttgggttgg

SEQ ID NO: 20 - DNA, 60 bp, Homo sapiens
  source 1..60: mol_type = genomic DNA
ggagcagccgggttggcctaagggaccttagtgctgggcggaaaggggactttgggttgg

SEQ ID NO: 21 - DNA, 30 bp, synthetic construct
  source 1..30: mol_type = other DNA
gcagtcgaacatgtagctgactcaggtcac

SEQ ID NO: 22 - DNA, 30 bp, synthetic construct
  source 1..30: mol_type = other DNA
tggatcacttgtgcaagcatcacatcgtag